European Patent Specification EP 3 662 053 B1, published September 25, 2024. Title: CRYPTIC METABOLITES AND METHOD FOR ACTIVATING SILENT BIOSYNTHETIC GENE CLUSTERS IN DIVERSE MICROORGANISMS. Applicant: The Trustees Of Princeton University. The sequence listing filed with the application follows.

SEQUENCE LISTING (1 sequence)

SEQ ID NO: 1 - protein, 14 aa, Streptomyces canus
GVGFPLADFFIHFD